European Patent Specification EP 3 492 600 B1, published April 24, 2024. Title: Method for measurement of the glycosylated hemoglobin. Applicant: KYOWA MEDEX CO.,LTD. The sequence listing filed with the application follows.

SEQUENCE LISTING (10 sequences)

SEQ ID NO: 1 - DNA, 1317 bp, Artificial Sequence
  FPOX-42
atggcgccccgagccaacaccaaaatcatcgtcgtcggcggcggcggcacaatgggctcgtcgacagccctacacctcctgcgcgccggctacacgccgtccaacatcacagtgctcgacacgtaccctatcccttccgcacagtctgcaggctacgacctgaacaagatcttcggcatctcaggcgcgaacaagcatgacttacaactctcgcttgaggcgttcgacatgtggaaaaatgatcctctattcaagccgtttttccacaatgttggacagatggacgtctcttcaacagaagaaggcatcaaacgccttcgccgcagataccagtctcttctccgcgcaggcattgggctcgagaagacgaatttcctgctggaaagtgaagacgagatcctggctaaagcgccgcatttcacgcgggagcagattaaaggctggaaagggctgttctgtggcgacggcggttggctcgctgcagccaaagccatcaatgccatcgggcagttcctcaaggaacagggcgtcaagtttggatttggcgaggccggcacgttcaaaaagccactcttcgccgatgccgacgagaagacgtgcatcggcgtcgaaactgtagacggcacaaaatactacgccgacaaggtcgttctagcagctggtgcctggagttcgacgttggtcgatctggaggagcagtgcgtttcaaaggcctgggtctttgcccacatccaactgacgcccgctgaagcagccgcgtacaagaacactcctgttatatacgacggtgactatgggtttttcattgagccggacgagaacggcatcataaaagtctgcgacgaattccctggcttcacgcacttcaagatgcaccagccgtacggctcaccggtgcccaaattgatctctgtgcctcgctcccatgcgaagcaccccacagatacatacccgcacgcgtcggaggtcaccatcaaaaaggctatcaaccggttcctgccgaggttcaatgacaaggaactgtttaacagggccatgtgctggtgcaccgataccgcggatagcaatctgcttgtttgtgagcatccacgctggaaggggttttatcttgcaacaggggacagcgggcattcgttcaagttgctgccgaatattggaaagcacgttgtcgagttattggaggggaggctggaaagtgtgtttaaggatgcttggaggtggaggcctggcagtggggatgcattaaagagtagacgggctgcgcctgcgaaggacctggcggatatgccggggtggaggaatgaggcaaagatgtag

SEQ ID NO: 2 - DNA, 31 bp, Artificial Sequence
  FPOX-42 F342V-F
gaggttcaatgacaaggaactggtgaacagg

SEQ ID NO: 3 - DNA, 30 bp, Artificial Sequence
  FPOX-42 F342V-R
gcaccagcacatggccctgttcaccagttc

SEQ ID NO: 4 - DNA, 1317 bp, Artificial Sequence
  FPOX-47
atggcgccccgagccaacaccaaaatcatcgtcgtcggcggcggcggcacaatgggctcgtcgacagccctacacctcctgcgcgccggctacacgccgtccaacatcacagtgctcgacacgtaccctatcccttccgcacagtctgcaggctacgacctgaacaagatcttcggcatctcaggcgcgaacaagcatgacttacaactctcgcttgaggcgttcgacatgtggaaaaatgatcctctattcaagccgtttttccacaatgttggacagatggacgtctcttcaacagaagaaggcatcaaacgccttcgccgcagataccagtctcttctccgcgcaggcattgggctcgagaagacgaatttcctgctggaaagtgaagacgagatcctggctaaagcgccgcatttcacgcgggagcagattaaaggctggaaagggctgttctgtggcgacggcggttggctcgctgcagccaaagccatcaatgccatcgggcagttcctcaaggaacagggcgtcaagtttggatttggcgaggccggcacgttcaaaaagccactcttcgccgatgccgacgagaagacgtgcatcggcgtcgaaactgtagacggcacaaaatactacgccgacaaggtcgttctagcagctggtgcctggagttcgacgttggtcgatctggaggagcagtgcgtttcaaaggcctgggtctttgcccacatccaactgacgcccgctgaagcagccgcgtacaagaacactcctgttatatacgacggtgactatgggtttttcattgagccggacgagaacggcatcataaaagtctgcgacgaattccctggcttcacgcacttcaagatgcaccagccgtacggctcaccggtgcccaaattgatctctgtgcctcgctcccatgcgaagcaccccacagatacatacccgcacgcgtcggaggtcaccatcaaaaaggctatcaaccggttcctgccgaggttcaatgacaaggaactggtgaacagggccatgtgctggtgcaccgataccgcggatagcaatctgcttgtttgtgagcatccacgctggaaggggttttatcttgcaacaggggacagcgggcattcgttcaagttgctgccgaatattggaaagcacgttgtcgagttattggaggggaggctggaaagtgtgtttaaggatgcttggaggtggaggcctggcagtggggatgcattaaagagtagacgggctgcgcctgcgaaggacctggcggatatgccggggtggaggaatgaggcaaagatgtag

SEQ ID NO: 5 - DNA, 21 bp, Artificial Sequence
  pTrc-F
caattaatcatccggctcgta

SEQ ID NO: 6 - DNA, 20 bp, Artificial Sequence
  pTrc-R
cttctgagttcggcatgggg

SEQ ID NO: 7 - DNA, 39 bp, Artificial Sequence
  FPOX-47 ¢3-R
atgggatccctactcattcctccaccccggcatatccgc

SEQ ID NO: 8 - DNA, 1308 bp, Artificial Sequence
  FPOX-47 ¢3
atggcgccccgagccaacaccaaaatcatcgtcgtcggcggcggcggcacaatgggctcgtcgacagccctacacctcctgcgcgccggctacacgccgtccaacatcacagtgctcgacacgtaccctatcccttccgcacagtctgcaggctacgacctgaacaagatcttcggcatctcaggcgcgaacaagcatgacttacaactctcgcttgaggcgttcgacatgtggaaaaatgatcctctattcaagccgtttttccacaatgttggacagatggacgtctcttcaacagaagaaggcatcaaacgccttcgccgcagataccagtctcttctccgcgcaggcattgggctcgagaagacgaatttcctgctggaaagtgaagacgagatcctggctaaagcgccgcatttcacgcgggagcagattaaaggctggaaagggctgttctgtggcgacggcggttggctcgctgcagccaaagccatcaatgccatcgggcagttcctcaaggaacagggcgtcaagtttggatttggcgaggccggcacgttcaaaaagccactcttcgccgatgccgacgagaagacgtgcatcggcgtcgaaactgtagacggcacaaaatactacgccgacaaggtcgttctagcagctggtgcctggagttcgacgttggtcgatctggaggagcagtgcgtttcaaaggcctgggtctttgcccacatccaactgacgcccgctgaagcagccgcgtacaagaacactcctgttatatacgacggtgactatgggtttttcattgagccggacgagaacggcatcataaaagtctgcgacgaattccctggcttcacgcacttcaagatgcaccagccgtacggctcaccggtgcccaaattgatctctgtgcctcgctcccatgcgaagcaccccacagatacatacccgcacgcgtcggaggtcaccatcaaaaaggctatcaaccggttcctgccgaggttcaatgacaaggaactggtgaacagggccatgtgctggtgcaccgataccgcggatagcaatctgcttgtttgtgagcatccacgctggaaggggttttatcttgcaacaggggacagcgggcattcgttcaagttgctgccgaatattggaaagcacgttgtcgagttattggaggggaggctggaaagtgtgtttaaggatgcttggaggtggaggcctggcagtggggatgcattaaagagtagacgggctgcgcctgcgaaggacctggcggatatgccggggtggaggaatgagtag

SEQ ID NO: 9 - protein, 438 aa, Artificial Sequence
  FPOX-47
MAPRANTKIIVVGGGGTMGSSTALHLLRAGYTPSNITVLDTYPIPSAQSAGYDLNKIFGISGANKHDLQLSLEAFDMWKNDPLFKPFFHNVGQMDVSSTEEGIKRLRRRYQSLLRAGIGLEKTNFLLESEDEILAKAPHFTREQIKGWKGLFCGDGGWLAAAKAINAIGQFLKEQGVKFGFGEAGTFKKPLFADADEKTCIGVETVDGTKYYADKVVLAAGAWSSTLVDLEEQCVSKAWVFAHIQLTPAEAAAYKNTPVIYDGDYGFFIEPDENGIIKVCDEFPGFTHFKMHQPYGSPVPKLISVPRSHAKHPTDTYPHASEVTIKKAINRFLPRFNDKELVNRAMCWCTDTADSNLLVCEHPRWKGFYLATGDSGHSFKLLPNIGKHVVELLEGRLESVFKDAWRWRPGSGDALKSRRAAPAKDLADMPGWRNEAKM

SEQ ID NO: 10 - protein, 435 aa, Artificial Sequence
  FPOX-47 ¢3
MAPRANTKIIVVGGGGTMGSSTALHLLRAGYTPSNITVLDTYPIPSAQSAGYDLNKIFGISGANKHDLQLSLEAFDMWKNDPLFKPFFHNVGQMDVSSTEEGIKRLRRRYQSLLRAGIGLEKTNFLLESEDEILAKAPHFTREQIKGWKGLFCGDGGWLAAAKAINAIGQFLKEQGVKFGFGEAGTFKKPLFADADEKTCIGVETVDGTKYYADKVVLAAGAWSSTLVDLEEQCVSKAWVFAHIQLTPAEAAAYKNTPVIYDGDYGFFIEPDENGIIKVCDEFPGFTHFKMHQPYGSPVPKLISVPRSHAKHPTDTYPHASEVTIKKAINRFLPRFNDKELVNRAMCWCTDTADSNLLVCEHPRWKGFYLATGDSGHSFKLLPNIGKHVVELLEGRLESVFKDAWRWRPGSGDALKSRRAAPAKDLADMPGWRNE